European Patent Application EP 4 438 737 A1, published October 2, 2024. Title: A method of quantifying a concentration of an analyte in a sample. Applicant: BLINK AG. The sequence listing filed with the application follows.

SEQUENCE LISTING (6 sequences)

SEQ ID NO: 1 - DNA, 22 bp, synthetic construct
  source 1..22: mol_type = other DNA
  misc_feature 1..22: note = forward primer sequence for human RPP30
gccaaattctgctcgttgttag

SEQ ID NO: 2 - DNA, 22 bp, synthetic construct
  source 1..22: mol_type = other DNA
  misc_feature 1..22: note = reverse primer sequence for human RPP30
cttccctcacggcatatacttc

SEQ ID NO: 3 - DNA, 24 bp, synthetic construct
  source 1..24: mol_type = other DNA
  misc_feature 1..24: note = probe sequence for human RPP30
  misc_feature 1: note = /note = Atto488-label
  misc_feature 24: note = /note = BHQ-1-label
tcaccagctggatgtccacattca

SEQ ID NO: 4 - DNA, 125 bp, synthetic construct
  source 1..125: mol_type = other DNA
  misc_feature 1..125: note = DNA label to be coupled to cTnI detection antibody
gcgtcagaccccgtagaaaagatcaaaggatcttcttgagatcctttttttctgcgcgtaatctgctgcttgcaaacaaaaaaaccaccgctaccagcggtggtttgtttgccggatcaagagct

SEQ ID NO: 5 - DNA, 20 bp, synthetic construct
  source 1..20: mol_type = other DNA
  misc_feature 1..20: note = forward primer for detection of labeled detection antibodies
agctcttgatccggcaaaca

SEQ ID NO: 6 - DNA, 20 bp, synthetic construct
  source 1..20: mol_type = other DNA
  misc_feature 1..20: note = reverse primer for detection of labeled detection antibodies
gcgtcagaccccgtagaaaa